European Patent Application EP 4 299 765 A1, published January 3, 2024. Title: Nucleic acid detection and quantification methods from environmental samples. Applicant: NATIONAL UNIVERSITY CORPORATION HOKKAIDO UNIVERSITY SHIONOGI & CO., LTD. The sequence listing filed with the application follows.

SEQUENCE LISTING (7 sequences)

SEQ ID NO: 1 - DNA, 20 bp, Artificial sequence
  Forward Primer
gaccccaaaatcagcgaaat

SEQ ID NO: 2 - DNA, 24 bp, Artificial sequence
  Reverse Primer
tctggttactgccagttgaatctg

SEQ ID NO: 3 - DNA, 24 bp, Artificial sequence
  Probe
accccgcattacgtttggtggacc

SEQ ID NO: 4 - DNA, 24 bp, Artificial sequence
  Forward primer
gagtggtttgaccttaacgtttga

SEQ ID NO: 5 - DNA, 20 bp, Artificial sequence
  Reverse primer
ttgtcggttgcaatgcaagt

SEQ ID NO: 6 - DNA, 16 bp, Artificial sequence
  Probe
cctaccgaagcaaatg

SEQ ID NO: 7 - DNA, 68 bp, Artificial sequence
  plasmid DNA
gagtggtttgaccttaacgtttgagaggcctaccgaagcaaatgtcgcacttgcattgcaaccgacaa